European Patent Specification EP 4 023 641 B1, published May 1, 2024. Title: METHOD OF SYNTHESIZING THYROID HORMONE ANALOGS AND POLYMORPHS THEREOF. Applicant: F. Hoffmann-La Roche Ltd. Madrigal Pharmaceuticals, Inc. Application EP 13 837 402.0. The sequence listing filed with the application follows.

SEQUENCE LISTING (2 sequences)

SEQ ID NO: 1 - protein, 259 aa, Homo sapiens
ELQKSIGHKPEPTDEEWELIKTVTEAHVATNAQGSHWKQKRKFLPEDIGQAPIVNAPEGGKVDLEAFSHFTKIITPAITRVVDFAKKLPMFCELPCEDQIILLKGCCMEIMSLRAAVRYDPESETLTLNGEMAVTRGQLKNGGLGVVSDAIFDLGMSLSSFNLDDTEVALLQAVLLMSSDRPGLACVERIEKYQDSFLLAFEHYINYRKHHVTHFWPKLLMKVTDLRMIGACHASRFLHMKVECPTELFPPLFLEVFED

SEQ ID NO: 2 - DNA, 780 bp, Homo sapiens
gagctgcagaagtccatcgggcacaagccagagcccacagacgaggaatgggagctcatcaaaactgtcaccgaagcccatgtggcgaccaacgcccaaggcagccactggaagcaaaaacggaaattcctgccagaagacattggacaagcaccaatagtcaatgccccagaaggtggaaaggttgacttggaagccttcagccattttacaaaaatcatcacaccagcaattaccagagtggtggattttgccaaaaagttgcctatgttttgtgagctgccatgtgaagaccagatcatcctcctcaaaggctgctgcatggagatcatgtcccttcgcgctgctgtgcgctatgacccagaaagtgagactttaaccttgaatggggaaatggcagtgacacggggccagctgaaaaatgggggtcttggggtggtgtcagacgccatctttgacctgggcatgtctctgtcttctttcaacctggatgacactgaagtagccctccttcaggccgtcctgctgatgtcttcagatcgcccggggcttgcctgtgttgagagaatagaaaagtaccaagatagtttcctgctggcctttgaacactatatcaattaccgaaaacaccacgtgacacacttttggccaaaactcctgatgaaggtgacagatctgcggatgataggagcctgccatgccagccgcttcctgcacatgaaggtggaatgccccacagaactcttcccccctttgttcttggaagtgttcgaggattag